European Patent Application EP 4 541 374 A2, published April 23, 2025. Title: DEFINED MULTI-CONJUGATE OLIGONUCLEOTIDES. Applicant: MPEG LA, L.L.C. Application EP. The sequence listing filed with the application follows.

SEQUENCE LISTING (164 sequences)

SEQ ID NO: 1 - DNA, 20 bp, synthetic construct
  misc_feature 1..20: note = Description of Artificial Sequence: Synthetic oligonucleotide
  misc_feature 1..20: note = Description of Combined DNA/RNA Molecule: Synthetic oligonucleotide
  source 1..20: mol_type = other DNA
gcaaaggcgtgccaactcat

SEQ ID NO: 2 - DNA, 20 bp, synthetic construct
  misc_feature 1..20: note = Description of Artificial Sequence: Synthetic oligonucleotide
  misc_feature 1..20: note = Description of Combined DNA/RNA Molecule: Synthetic oligonucleotide
  source 1..20: mol_type = other DNA
gcaaaggcgtgccaactcat

SEQ ID NO: 3 - DNA, 20 bp, synthetic construct
  misc_feature 1..20: note = Description of Artificial Sequence: Synthetic oligonucleotide
  misc_feature 1..20: note = Description of Combined DNA/RNA Molecule: Synthetic oligonucleotide
  source 1..20: mol_type = other DNA
gcaaaggcgtgccaactcat

SEQ ID NO: 4 - DNA, 20 bp, synthetic construct
  misc_feature 1..20: note = Description of Artificial Sequence: Synthetic oligonucleotide
  misc_feature 1..20: note = Description of Combined DNA/RNA Molecule: Synthetic oligonucleotide
  source 1..20: mol_type = other DNA
gcaaaggcgtgccaactcat

SEQ ID NO: 5 - DNA, 20 bp, synthetic construct
  misc_feature 1..20: note = Description of Artificial Sequence: Synthetic oligonucleotide
  misc_feature 1..20: note = Description of Combined DNA/RNA Molecule: Synthetic oligonucleotide
  source 1..20: mol_type = other DNA
gcaaaggcgtgccaactcat

SEQ ID NO: 6 - DNA, 20 bp, synthetic construct
  misc_feature 1..20: note = Description of Artificial Sequence: Synthetic oligonucleotide
  misc_feature 1..20: note = Description of Combined DNA/RNA Molecule: Synthetic oligonucleotide
  source 1..20: mol_type = other DNA
gcaaaggcgtgccaactcat

SEQ ID NO: 7 - DNA, 22 bp, synthetic construct
  misc_feature 1..22: note = Description of Artificial Sequence: Synthetic oligonucleotide
  misc_feature 1..22: note = Description of Combined DNA/RNA Molecule: Synthetic oligonucleotide
  source 1..22: mol_type = other DNA
tgagttggcacgcctttgcttt

SEQ ID NO: 8 - RNA, 21 nt, synthetic construct
  modified_base 1: mod_base = OTHER; note = thymine
  modified_base 5..6: mod_base = OTHER; note = thymine
  modified_base 15..17: mod_base = OTHER; note = thymine
  modified_base 20..21: mod_base = OTHER; note = thymine
  misc_feature 1..21: note = Description of Artificial Sequence: Synthetic oligonucleotide
  source 1..21: mol_type = other RNA
tgagttggcacgcctttgctt

SEQ ID NO: 9 - RNA, 21 nt, synthetic construct
  modified_base 1: mod_base = OTHER; note = thymine
  modified_base 5..6: mod_base = OTHER; note = thymine
  modified_base 15..17: mod_base = OTHER; note = thymine
  modified_base 20..21: mod_base = OTHER; note = thymine
  misc_feature 1..21: note = Description of Artificial Sequence: Synthetic oligonucleotide
  source 1..21: mol_type = other RNA
tgagttggcacgcctttgctt

SEQ ID NO: 10 - DNA, 20 bp, synthetic construct
  misc_feature 1..20: note = Description of Artificial Sequence: Synthetic oligonucleotide
  misc_feature 1..20: note = Description of Combined DNA/RNA Molecule: Synthetic oligonucleotide
  source 1..20: mol_type = other DNA
ctatttggagagaaatcgat

SEQ ID NO: 11 - DNA, 20 bp, synthetic construct
  misc_feature 1..20: note = Description of Artificial Sequence: Synthetic oligonucleotide
  misc_feature 1..20: note = Description of Combined DNA/RNA Molecule: Synthetic oligonucleotide
  source 1..20: mol_type = other DNA
ctatttggagagaaatcgat

SEQ ID NO: 12 - DNA, 20 bp, synthetic construct
  misc_feature 1..20: note = Description of Artificial Sequence: Synthetic oligonucleotide
  misc_feature 1..20: note = Description of Combined DNA/RNA Molecule: Synthetic oligonucleotide
  source 1..20: mol_type = other DNA
ctatttggagagaaatcgat

SEQ ID NO: 13 - DNA, 21 bp, synthetic construct
  misc_feature 1..21: note = Description of Artificial Sequence: Synthetic oligonucleotide
  misc_feature 1..21: note = Description of Combined DNA/RNA Molecule: Synthetic oligonucleotide
  source 1..21: mol_type = other DNA
ggatcatctcaagtcttactt

SEQ ID NO: 14 - DNA, 21 bp, synthetic construct
  misc_feature 1..21: note = Description of Artificial Sequence: Synthetic oligonucleotide
  misc_feature 1..21: note = Description of Combined DNA/RNA Molecule: Synthetic oligonucleotide
  source 1..21: mol_type = other DNA
gtaagacttgagatgatcctt

SEQ ID NO: 15 - skipped

SEQ ID NO: 16 - DNA, 21 bp, synthetic construct
  misc_feature 1..21: note = Description of Artificial Sequence: Synthetic oligonucleotide
  misc_feature 1..21: note = Description of Combined DNA/RNA Molecule: Synthetic oligonucleotide
  source 1..21: mol_type = other DNA
gcaaaggcgtgccaactcatt

SEQ ID NO: 17 - DNA, 21 bp, synthetic construct
  misc_feature 1..21: note = Description of Artificial Sequence: Synthetic oligonucleotide
  misc_feature 1..21: note = Description of Combined DNA/RNA Molecule: Synthetic oligonucleotide
  source 1..21: mol_type = other DNA
tgagttggcacgcctttgctt

SEQ ID NO: 18 - skipped

SEQ ID NO: 19 - RNA, 21 nt, synthetic construct
  modified_base 5: mod_base = OTHER; note = thymine
  modified_base 7..8: mod_base = OTHER; note = thymine
  modified_base 10: mod_base = OTHER; note = thymine
  modified_base 12..14: mod_base = OTHER; note = thymine
  modified_base 17: mod_base = OTHER; note = thymine
  misc_feature 1..21: note = Description of Artificial Sequence: Synthetic oligonucleotide
  source 1..21: mol_type = other RNA
ggaatcttatatttgatccaa

SEQ ID NO: 20 - RNA, 23 nt, synthetic construct
  modified_base 1..2: mod_base = OTHER; note = thymine
  modified_base 6: mod_base = OTHER; note = thymine
  modified_base 11: mod_base = OTHER; note = thymine
  modified_base 13: mod_base = OTHER; note = thymine
  modified_base 18..19: mod_base = OTHER; note = thymine
  modified_base 23: mod_base = OTHER; note = thymine
  misc_feature 1..23: note = Description of Artificial Sequence: Synthetic oligonucleotide
  source 1..23: mol_type = other RNA
ttggatcaaatataagattccct

SEQ ID NO: 21 - skipped

SEQ ID NO: 22 - DNA, 21 bp, synthetic construct
  misc_feature 1..21: note = Description of Artificial Sequence: Synthetic oligonucleotide
  misc_feature 1..21: note = Description of Combined DNA/RNA Molecule: Synthetic oligonucleotide
  source 1..21: mol_type = other DNA
cttacgctgagtacttcgatt

SEQ ID NO: 23 - DNA, 21 bp, synthetic construct
  misc_feature 1..21: note = Description of Artificial Sequence: Synthetic oligonucleotide
  misc_feature 1..21: note = Description of Combined DNA/RNA Molecule: Synthetic oligonucleotide
  source 1..21: mol_type = other DNA
tcgaagtactcagcgtaagtt

SEQ ID NO: 24 - skipped

SEQ ID NO: 25 - DNA, 20 bp, synthetic construct
  misc_feature 1..20: note = Description of Artificial Sequence: Synthetic oligonucleotide
  misc_feature 1..20: note = Description of Combined DNA/RNA Molecule: Synthetic oligonucleotide
  source 1..20: mol_type = other DNA
gcaaaggcgtgccaactcat

SEQ ID NO: 26 - RNA, 21 nt, synthetic construct
  modified_base 1: mod_base = OTHER; note = thymine
  modified_base 5..6: mod_base = OTHER; note = thymine
  modified_base 15..17: mod_base = OTHER; note = thymine
  modified_base 20..21: mod_base = OTHER; note = thymine
  misc_feature 1..21: note = Description of Artificial Sequence: Synthetic oligonucleotide
  source 1..21: mol_type = other RNA
tgagttggcacgcctttgctt

SEQ ID NO: 27 - skipped

SEQ ID NO: 28 - DNA, 20 bp, synthetic construct
  misc_feature 1..20: note = Description of Artificial Sequence: Synthetic oligonucleotide
  misc_feature 1..20: note = Description of Combined DNA/RNA Molecule: Synthetic oligonucleotide
  source 1..20: mol_type = other DNA
ctatttggagagaaatcgat

SEQ ID NO: 29 - RNA, 21 nt, synthetic construct
  modified_base 1: mod_base = OTHER; note = thymine
  modified_base 5..7: mod_base = OTHER; note = thymine
  modified_base 9: mod_base = OTHER; note = thymine
  modified_base 11: mod_base = OTHER; note = thymine
  modified_base 17: mod_base = OTHER; note = thymine
  modified_base 20..21: mod_base = OTHER; note = thymine
  misc_feature 1..21: note = Description of Artificial Sequence: Synthetic oligonucleotide
  source 1..21: mol_type = other RNA
tcgatttctctccaaatagtt

SEQ ID NO: 30 - skipped

SEQ ID NO: 31 - DNA, 22 bp, synthetic construct
  misc_feature 1..22: note = Description of Artificial Sequence: Synthetic oligonucleotide
  misc_feature 1..22: note = Description of Combined DNA/RNA Molecule: Synthetic oligonucleotide
  source 1..22: mol_type = other DNA
aacagtgttcttgctctataat

SEQ ID NO: 32 - RNA, 23 nt, synthetic construct
  modified_base 1..2: mod_base = OTHER; note = thymine
  modified_base 4: mod_base = OTHER; note = thymine
  modified_base 18: mod_base = OTHER; note = thymine
  modified_base 20..23: mod_base = OTHER; note = thymine
  misc_feature 1..23: note = Description of Artificial Sequence: Synthetic oligonucleotide
  source 1..23: mol_type = other RNA
ttatagagcaagaacactgtttt

SEQ ID NO: 33 - skipped

SEQ ID NO: 34 - DNA, 20 bp, synthetic construct
  misc_feature 1..20: note = Description of Artificial Sequence: Synthetic oligonucleotide
  misc_feature 1..20: note = Description of Combined DNA/RNA Molecule: Synthetic oligonucleotide
  source 1..20: mol_type = other DNA
gcaaaggcgtgccaactcat

SEQ ID NO: 35 - DNA, 20 bp, synthetic construct
  misc_feature 1..20: note = Description of Artificial Sequence: Synthetic oligonucleotide
  misc_feature 1..20: note = Description of Combined DNA/RNA Molecule: Synthetic oligonucleotide
  source 1..20: mol_type = other DNA
gcaaaggcgtgccaactcat

SEQ ID NO: 36 - skipped

SEQ ID NO: 37 - RNA, 21 nt, synthetic construct
  modified_base 5: mod_base = OTHER; note = thymine
  modified_base 7..8: mod_base = OTHER; note = thymine
  modified_base 10: mod_base = OTHER; note = thymine
  modified_base 12..14: mod_base = OTHER; note = thymine
  modified_base 17: mod_base = OTHER; note = thymine
  misc_feature 1..21: note = Description of Artificial Sequence: Synthetic oligonucleotide
  source 1..21: mol_type = other RNA
ggaatcttatatttgatccaa

SEQ ID NO: 38 - DNA, 21 bp, synthetic construct
  misc_feature 1..21: note = Description of Artificial Sequence: Synthetic oligonucleotide
  misc_feature 1..21: note = Description of Combined DNA/RNA Molecule: Synthetic oligonucleotide
  source 1..21: mol_type = other DNA
ggatcatctcaagtcttactt

SEQ ID NO: 39 - DNA, 20 bp, synthetic construct
  misc_feature 1..20: note = Description of Artificial Sequence: Synthetic oligonucleotide
  misc_feature 1..20: note = Description of Combined DNA/RNA Molecule: Synthetic oligonucleotide
  source 1..20: mol_type = other DNA
gcaaaggcgtgccaactcat

SEQ ID NO: 40 - RNA, 21 nt, synthetic construct
  modified_base 1: mod_base = OTHER; note = thymine
  modified_base 5..6: mod_base = OTHER; note = thymine
  modified_base 15..17: mod_base = OTHER; note = thymine
  modified_base 20..21: mod_base = OTHER; note = thymine
  misc_feature 1..21: note = Description of Artificial Sequence: Synthetic oligonucleotide
  source 1..21: mol_type = other RNA
tgagttggcacgcctttgctt

SEQ ID NO: 41 - DNA, 20 bp, synthetic construct
  misc_feature 1..20: note = Description of Artificial Sequence: Synthetic oligonucleotide
  misc_feature 1..20: note = Description of Combined DNA/RNA Molecule: Synthetic oligonucleotide
  source 1..20: mol_type = other DNA
gcaaaggcgtgccaactcat

SEQ ID NO: 42-43 - skipped (2 entries)

SEQ ID NO: 44 - RNA, 23 nt, synthetic construct
  modified_base 1..2: mod_base = OTHER; note = thymine
  modified_base 4: mod_base = OTHER; note = thymine
  modified_base 18: mod_base = OTHER; note = thymine
  modified_base 20..23: mod_base = OTHER; note = thymine
  misc_feature 1..23: note = Description of Artificial Sequence: Synthetic oligonucleotide
  source 1..23: mol_type = other RNA
ttatagagcaagaacactgtttt

SEQ ID NO: 45 - DNA, 22 bp, synthetic construct
  misc_feature 1..22: note = Description of Artificial Sequence: Synthetic oligonucleotide
  misc_feature 1..22: note = Description of Combined DNA/RNA Molecule: Synthetic oligonucleotide
  source 1..22: mol_type = other DNA
aacagtgttcttgctctataat

SEQ ID NO: 46 - DNA, 20 bp, synthetic construct
  misc_feature 1..20: note = Description of Artificial Sequence: Synthetic oligonucleotide
  misc_feature 1..20: note = Description of Combined DNA/RNA Molecule: Synthetic oligonucleotide
  source 1..20: mol_type = other DNA
gcaaaggcgtgccaactcat

SEQ ID NO: 47 - RNA, 23 nt, synthetic construct
  modified_base 1..2: mod_base = OTHER; note = thymine
  modified_base 4: mod_base = OTHER; note = thymine
  modified_base 18: mod_base = OTHER; note = thymine
  modified_base 20..23: mod_base = OTHER; note = thymine
  misc_feature 1..23: note = Description of Artificial Sequence: Synthetic oligonucleotide
  source 1..23: mol_type = other RNA
ttatagagcaagaacactgtttt

SEQ ID NO: 48 - DNA, 22 bp, synthetic construct
  misc_feature 1..22: note = Description of Artificial Sequence: Synthetic oligonucleotide
  misc_feature 1..22: note = Description of Combined DNA/RNA Molecule: Synthetic oligonucleotide
  source 1..22: mol_type = other DNA
aacagtgttcttgctctataat

SEQ ID NO: 49-51 - skipped (3 entries)

SEQ ID NO: 52 - DNA, 20 bp, synthetic construct
  misc_feature 1..20: note = Description of Artificial Sequence: Synthetic oligonucleotide
  misc_feature 1..20: note = Description of Combined DNA/RNA Molecule: Synthetic oligonucleotide
  source 1..20: mol_type = other DNA
gcaaaggcgtgccaactcat

SEQ ID NO: 53-55 - skipped (3 entries)

SEQ ID NO: 56 - DNA, 21 bp, synthetic construct
  misc_feature 1..21: note = Description of Artificial Sequence: Synthetic oligonucleotide
  misc_feature 1..21: note = Description of Combined DNA/RNA Molecule: Synthetic oligonucleotide
  source 1..21: mol_type = other DNA
ggatcatctcaagtcttactt

SEQ ID NO: 57 - DNA, 21 bp, synthetic construct
  misc_feature 1..21: note = Description of Artificial Sequence: Synthetic oligonucleotide
  misc_feature 1..21: note = Description of Combined DNA/RNA Molecule: Synthetic oligonucleotide
  source 1..21: mol_type = other DNA
gtaagacttgagatgatcctt

SEQ ID NO: 58 - DNA, 21 bp, synthetic construct
  misc_feature 1..21: note = Description of Artificial Sequence: Synthetic oligonucleotide
  misc_feature 1..21: note = Description of Combined DNA/RNA Molecule: Synthetic oligonucleotide
  source 1..21: mol_type = other DNA
ggatcatctcaagtcttactt

SEQ ID NO: 59 - DNA, 21 bp, synthetic construct
  misc_feature 1..21: note = Description of Artificial Sequence: Synthetic oligonucleotide
  misc_feature 1..21: note = Description of Combined DNA/RNA Molecule: Synthetic oligonucleotide
  source 1..21: mol_type = other DNA
gtaagacttgagatgatcctt

SEQ ID NO: 60 - DNA, 21 bp, synthetic construct
  misc_feature 1..21: note = Description of Artificial Sequence: Synthetic oligonucleotide
  misc_feature 1..21: note = Description of Combined DNA/RNA Molecule: Synthetic oligonucleotide
  source 1..21: mol_type = other DNA
ggatcatctcaagtcttactt

SEQ ID NO: 61 - DNA, 21 bp, synthetic construct
  misc_feature 1..21: note = Description of Artificial Sequence: Synthetic oligonucleotide
  misc_feature 1..21: note = Description of Combined DNA/RNA Molecule: Synthetic oligonucleotide
  source 1..21: mol_type = other DNA
gtaagacttgagatgatcctt

SEQ ID NO: 62-64 - skipped (3 entries)

SEQ ID NO: 65 - RNA, 19 nt, synthetic construct
  modified_base 8: mod_base = OTHER; note = thymine
  modified_base 10: mod_base = OTHER; note = thymine
  modified_base 15..16: mod_base = OTHER; note = thymine
  misc_feature 1..19: note = Description of Artificial Sequence: Synthetic oligonucleotide
  source 1..19: mol_type = other RNA
caaccagtgtacccttaaa

SEQ ID NO: 66 - RNA, 19 nt, synthetic construct
  modified_base 2: mod_base = OTHER; note = thymine
  modified_base 4: mod_base = OTHER; note = thymine
  modified_base 6: mod_base = OTHER; note = thymine
  modified_base 13: mod_base = OTHER; note = thymine
  misc_feature 1..19: note = Description of Artificial Sequence: Synthetic oligonucleotide
  source 1..19: mol_type = other RNA
ctgtgtacgaagtacaaaa

SEQ ID NO: 67 - RNA, 19 nt, synthetic construct
  modified_base 6: mod_base = OTHER; note = thymine
  modified_base 8: mod_base = OTHER; note = thymine
  modified_base 13: mod_base = OTHER; note = thymine
  modified_base 16: mod_base = OTHER; note = thymine
  misc_feature 1..19: note = Description of Artificial Sequence: Synthetic oligonucleotide
  source 1..19: mol_type = other RNA
caacctatgaactcctaaa

SEQ ID NO: 68 - RNA, 19 nt, synthetic construct
  modified_base 3..4: mod_base = OTHER; note = thymine
  modified_base 10: mod_base = OTHER; note = thymine
  modified_base 17..19: mod_base = OTHER; note = thymine
  misc_feature 1..19: note = Description of Artificial Sequence: Synthetic oligonucleotide
  source 1..19: mol_type = other RNA
gcttacggctcaacaattt

SEQ ID NO: 69 - RNA, 19 nt, synthetic construct
  modified_base 6: mod_base = OTHER; note = thymine
  modified_base 9: mod_base = OTHER; note = thymine
  modified_base 14: mod_base = OTHER; note = thymine
  modified_base 16: mod_base = OTHER; note = thymine
  misc_feature 1..19: note = Description of Artificial Sequence: Synthetic oligonucleotide
  source 1..19: mol_type = other RNA
gcacgtgatggactatcaa

SEQ ID NO: 70 - RNA, 19 nt, synthetic construct
  modified_base 2: mod_base = OTHER; note = thymine
  modified_base 4..6: mod_base = OTHER; note = thymine
  modified_base 16: mod_base = OTHER; note = thymine
  misc_feature 1..19: note = Description of Artificial Sequence: Synthetic oligonucleotide
  source 1..19: mol_type = other RNA
ctatttggagagaaatcga

SEQ ID NO: 71 - RNA, 19 nt, synthetic construct
  modified_base 5..6: mod_base = OTHER; note = thymine
  modified_base 8..9: mod_base = OTHER; note = thymine
  modified_base 12: mod_base = OTHER; note = thymine
  modified_base 17: mod_base = OTHER; note = thymine
  misc_feature 1..19: note = Description of Artificial Sequence: Synthetic oligonucleotide
  source 1..19: mol_type = other RNA
gagattattgatcgaatca

SEQ ID NO: 72 - RNA, 19 nt, synthetic construct
  modified_base 4: mod_base = OTHER; note = thymine
  modified_base 6: mod_base = OTHER; note = thymine
  modified_base 10: mod_base = OTHER; note = thymine
  modified_base 12: mod_base = OTHER; note = thymine
  misc_feature 1..19: note = Description of Artificial Sequence: Synthetic oligonucleotide
  source 1..19: mol_type = other RNA
ccgtgtaaatctagcaaaa

SEQ ID NO: 73 - RNA, 19 nt, synthetic construct
  modified_base 4..6: mod_base = OTHER; note = thymine
  modified_base 10: mod_base = OTHER; note = thymine
  modified_base 14..15: mod_base = OTHER; note = thymine
  misc_feature 1..19: note = Description of Artificial Sequence: Synthetic oligonucleotide
  source 1..19: mol_type = other RNA
gcatttagatcaattgaga

SEQ ID NO: 74 - RNA, 19 nt, synthetic construct
  modified_base 3..6: mod_base = OTHER; note = thymine
  modified_base 9: mod_base = OTHER; note = thymine
  modified_base 13: mod_base = OTHER; note = thymine
  modified_base 17: mod_base = OTHER; note = thymine
  misc_feature 1..19: note = Description of Artificial Sequence: Synthetic oligonucleotide
  source 1..19: mol_type = other RNA
ggttttaatggataaatca

SEQ ID NO: 75 - RNA, 19 nt, synthetic construct
  modified_base 4..6: mod_base = OTHER; note = thymine
  modified_base 16: mod_base = OTHER; note = thymine
  modified_base 18..19: mod_base = OTHER; note = thymine
  misc_feature 1..19: note = Description of Artificial Sequence: Synthetic oligonucleotide
  source 1..19: mol_type = other RNA
gactttgcagagcaatatt

SEQ ID NO: 76 - RNA, 19 nt, synthetic construct
  modified_base 2..3: mod_base = OTHER; note = thymine
  modified_base 9: mod_base = OTHER; note = thymine
  modified_base 12: mod_base = OTHER; note = thymine
  misc_feature 1..19: note = Description of Artificial Sequence: Synthetic oligonucleotide
  source 1..19: mol_type = other RNA
cttacgggtcatccaaaaa

SEQ ID NO: 77 - RNA, 19 nt, synthetic construct
  modified_base 1..3: mod_base = OTHER; note = thymine
  modified_base 9: mod_base = OTHER; note = thymine
  modified_base 14: mod_base = OTHER; note = thymine
  modified_base 17..18: mod_base = OTHER; note = thymine
  misc_feature 1..19: note = Description of Artificial Sequence: Synthetic oligonucleotide
  source 1..19: mol_type = other RNA
tttaagggtacactggttg

SEQ ID NO: 78 - RNA, 19 nt, synthetic construct
  modified_base 1..4: mod_base = OTHER; note = thymine
  modified_base 6: mod_base = OTHER; note = thymine
  modified_base 9..10: mod_base = OTHER; note = thymine
  modified_base 13: mod_base = OTHER; note = thymine
  misc_feature 1..19: note = Description of Artificial Sequence: Synthetic oligonucleotide
  source 1..19: mol_type = other RNA
ttttgtacttcgtacacag

SEQ ID NO: 79 - RNA, 19 nt, synthetic construct
  modified_base 1..3: mod_base = OTHER; note = thymine
  modified_base 9..10: mod_base = OTHER; note = thymine
  modified_base 13: mod_base = OTHER; note = thymine
  modified_base 17..18: mod_base = OTHER; note = thymine
  misc_feature 1..19: note = Description of Artificial Sequence: Synthetic oligonucleotide
  source 1..19: mol_type = other RNA
tttaggagttcataggttg

SEQ ID NO: 80 - RNA, 19 nt, synthetic construct
  modified_base 4..5: mod_base = OTHER; note = thymine
  modified_base 7..8: mod_base = OTHER; note = thymine
  modified_base 15: mod_base = OTHER; note = thymine
  misc_feature 1..19: note = Description of Artificial Sequence: Synthetic oligonucleotide
  source 1..19: mol_type = other RNA
aaattgttgagccgtaagc

SEQ ID NO: 81 - RNA, 19 nt, synthetic construct
  modified_base 1..2: mod_base = OTHER; note = thymine
  modified_base 5: mod_base = OTHER; note = thymine
  modified_base 8: mod_base = OTHER; note = thymine
  modified_base 12: mod_base = OTHER; note = thymine
  modified_base 17: mod_base = OTHER; note = thymine
  misc_feature 1..19: note = Description of Artificial Sequence: Synthetic oligonucleotide
  source 1..19: mol_type = other RNA
ttgatagtccatcacgtgc

SEQ ID NO: 82 - RNA, 19 nt, synthetic construct
  modified_base 1: mod_base = OTHER; note = thymine
  modified_base 5..7: mod_base = OTHER; note = thymine
  modified_base 9: mod_base = OTHER; note = thymine
  modified_base 11: mod_base = OTHER; note = thymine
  modified_base 17: mod_base = OTHER; note = thymine
  misc_feature 1..19: note = Description of Artificial Sequence: Synthetic oligonucleotide
  source 1..19: mol_type = other RNA
tcgatttctctccaaatag

SEQ ID NO: 83 - RNA, 19 nt, synthetic construct
  modified_base 1: mod_base = OTHER; note = thymine
  modified_base 4..5: mod_base = OTHER; note = thymine
  modified_base 9: mod_base = OTHER; note = thymine
  modified_base 13: mod_base = OTHER; note = thymine
  modified_base 16: mod_base = OTHER; note = thymine
  modified_base 18: mod_base = OTHER; note = thymine
  misc_feature 1..19: note = Description of Artificial Sequence: Synthetic oligonucleotide
  source 1..19: mol_type = other RNA
tgattcgatcaataatctc

SEQ ID NO: 84 - RNA, 19 nt, synthetic construct
  modified_base 1..4: mod_base = OTHER; note = thymine
  modified_base 7: mod_base = OTHER; note = thymine
  modified_base 11..13: mod_base = OTHER; note = thymine
  misc_feature 1..19: note = Description of Artificial Sequence: Synthetic oligonucleotide
  source 1..19: mol_type = other RNA
ttttgctagatttacacgg

SEQ ID NO: 85 - RNA, 19 nt, synthetic construct
  modified_base 1: mod_base = OTHER; note = thymine
  modified_base 3: mod_base = OTHER; note = thymine
  modified_base 7..8: mod_base = OTHER; note = thymine
  modified_base 11: mod_base = OTHER; note = thymine
  modified_base 13: mod_base = OTHER; note = thymine
  modified_base 17: mod_base = OTHER; note = thymine
  misc_feature 1..19: note = Description of Artificial Sequence: Synthetic oligonucleotide
  source 1..19: mol_type = other RNA
tctcaattgatctaaatgc

SEQ ID NO: 86 - RNA, 19 nt, synthetic construct
  modified_base 1: mod_base = OTHER; note = thymine
  modified_base 4..6: mod_base = OTHER; note = thymine
  modified_base 8: mod_base = OTHER; note = thymine
  modified_base 12..13: mod_base = OTHER; note = thymine
  misc_feature 1..19: note = Description of Artificial Sequence: Synthetic oligonucleotide
  source 1..19: mol_type = other RNA
tgatttatccattaaaacc

SEQ ID NO: 87 - RNA, 19 nt, synthetic construct
  modified_base 3: mod_base = OTHER; note = thymine
  modified_base 5..6: mod_base = OTHER; note = thymine
  modified_base 9: mod_base = OTHER; note = thymine
  modified_base 11: mod_base = OTHER; note = thymine
  modified_base 18: mod_base = OTHER; note = thymine
  misc_feature 1..19: note = Description of Artificial Sequence: Synthetic oligonucleotide
  source 1..19: mol_type = other RNA
aatattgctctgcaaagtc

SEQ ID NO: 88 - RNA, 19 nt, synthetic construct
  modified_base 1..5: mod_base = OTHER; note = thymine
  modified_base 9: mod_base = OTHER; note = thymine
  modified_base 16: mod_base = OTHER; note = thymine
  misc_feature 1..19: note = Description of Artificial Sequence: Synthetic oligonucleotide
  source 1..19: mol_type = other RNA
tttttggatgacccgtaag

SEQ ID NO: 89 - DNA, 21 bp, synthetic construct
  misc_feature 1..21: note = Description of Artificial Sequence: Synthetic oligonucleotide
  misc_feature 1..21: note = Description of Combined DNA/RNA Molecule: Synthetic oligonucleotide
  source 1..21: mol_type = other DNA
caaccagtgtacccttaaatt

SEQ ID NO: 90 - DNA, 21 bp, synthetic construct
  misc_feature 1..21: note = Description of Artificial Sequence: Synthetic oligonucleotide
  misc_feature 1..21: note = Description of Combined DNA/RNA Molecule: Synthetic oligonucleotide
  source 1..21: mol_type = other DNA
tttaagggtacactggttgtt

SEQ ID NO: 91 - skipped

SEQ ID NO: 92 - DNA, 21 bp, synthetic construct
  misc_feature 1..21: note = Description of Artificial Sequence: Synthetic oligonucleotide
  misc_feature 1..21: note = Description of Combined DNA/RNA Molecule: Synthetic oligonucleotide
  source 1..21: mol_type = other DNA
ctgtgtacgaagtacaaaatt

SEQ ID NO: 93 - DNA, 21 bp, synthetic construct
  misc_feature 1..21: note = Description of Artificial Sequence: Synthetic oligonucleotide
  misc_feature 1..21: note = Description of Combined DNA/RNA Molecule: Synthetic oligonucleotide
  source 1..21: mol_type = other DNA
ttttgtacttcgtacacagtt

SEQ ID NO: 94 - skipped

SEQ ID NO: 95 - DNA, 21 bp, synthetic construct
  misc_feature 1..21: note = Description of Artificial Sequence: Synthetic oligonucleotide
  misc_feature 1..21: note = Description of Combined DNA/RNA Molecule: Synthetic oligonucleotide
  source 1..21: mol_type = other DNA
caacctatgaactcctaaatt

SEQ ID NO: 96 - DNA, 21 bp, synthetic construct
  misc_feature 1..21: note = Description of Artificial Sequence: Synthetic oligonucleotide
  misc_feature 1..21: note = Description of Combined DNA/RNA Molecule: Synthetic oligonucleotide
  source 1..21: mol_type = other DNA
tttaggagttcataggttgtt

SEQ ID NO: 97 - skipped

SEQ ID NO: 98 - DNA, 21 bp, synthetic construct
  misc_feature 1..21: note = Description of Artificial Sequence: Synthetic oligonucleotide
  misc_feature 1..21: note = Description of Combined DNA/RNA Molecule: Synthetic oligonucleotide
  source 1..21: mol_type = other DNA
gcttacggctcaacaattttt

SEQ ID NO: 99 - DNA, 21 bp, synthetic construct
  misc_feature 1..21: note = Description of Artificial Sequence: Synthetic oligonucleotide
  misc_feature 1..21: note = Description of Combined DNA/RNA Molecule: Synthetic oligonucleotide
  source 1..21: mol_type = other DNA
aaattgttgagccgtaagctt

SEQ ID NO: 100 - skipped

SEQ ID NO: 101 - DNA, 21 bp, synthetic construct
  misc_feature 1..21: note = Description of Artificial Sequence: Synthetic oligonucleotide
  misc_feature 1..21: note = Description of Combined DNA/RNA Molecule: Synthetic oligonucleotide
  source 1..21: mol_type = other DNA
gcacgtgatggactatcaatt

SEQ ID NO: 102 - DNA, 21 bp, synthetic construct
  misc_feature 1..21: note = Description of Artificial Sequence: Synthetic oligonucleotide
  misc_feature 1..21: note = Description of Combined DNA/RNA Molecule: Synthetic oligonucleotide
  source 1..21: mol_type = other DNA
ttgatagtccatcacgtgctt

SEQ ID NO: 103 - skipped

SEQ ID NO: 104 - DNA, 21 bp, synthetic construct
  misc_feature 1..21: note = Description of Artificial Sequence: Synthetic oligonucleotide
  misc_feature 1..21: note = Description of Combined DNA/RNA Molecule: Synthetic oligonucleotide
  source 1..21: mol_type = other DNA
ctatttggagagaaatcgatt

SEQ ID NO: 105 - DNA, 21 bp, synthetic construct
  misc_feature 1..21: note = Description of Artificial Sequence: Synthetic oligonucleotide
  misc_feature 1..21: note = Description of Combined DNA/RNA Molecule: Synthetic oligonucleotide
  source 1..21: mol_type = other DNA
tcgatttctctccaaatagtt

SEQ ID NO: 106 - skipped

SEQ ID NO: 107 - DNA, 21 bp, synthetic construct
  misc_feature 1..21: note = Description of Artificial Sequence: Synthetic oligonucleotide
  misc_feature 1..21: note = Description of Combined DNA/RNA Molecule: Synthetic oligonucleotide
  source 1..21: mol_type = other DNA
gagattattgatcgaatcatt

SEQ ID NO: 108 - DNA, 21 bp, synthetic construct
  misc_feature 1..21: note = Description of Artificial Sequence: Synthetic oligonucleotide
  misc_feature 1..21: note = Description of Combined DNA/RNA Molecule: Synthetic oligonucleotide
  source 1..21: mol_type = other DNA
tgattcgatcaataatctctt

SEQ ID NO: 109 - skipped

SEQ ID NO: 110 - DNA, 21 bp, synthetic construct
  misc_feature 1..21: note = Description of Artificial Sequence: Synthetic oligonucleotide
  misc_feature 1..21: note = Description of Combined DNA/RNA Molecule: Synthetic oligonucleotide
  source 1..21: mol_type = other DNA
ccgtgtaaatctagcaaaatt

SEQ ID NO: 111 - DNA, 21 bp, synthetic construct
  misc_feature 1..21: note = Description of Artificial Sequence: Synthetic oligonucleotide
  misc_feature 1..21: note = Description of Combined DNA/RNA Molecule: Synthetic oligonucleotide
  source 1..21: mol_type = other DNA
ttttgctagatttacacggtt

SEQ ID NO: 112 - skipped

SEQ ID NO: 113 - DNA, 21 bp, synthetic construct
  misc_feature 1..21: note = Description of Artificial Sequence: Synthetic oligonucleotide
  misc_feature 1..21: note = Description of Combined DNA/RNA Molecule: Synthetic oligonucleotide
  source 1..21: mol_type = other DNA
gcatttagatcaattgagatt

SEQ ID NO: 114 - DNA, 21 bp, synthetic construct
  misc_feature 1..21: note = Description of Artificial Sequence: Synthetic oligonucleotide
  misc_feature 1..21: note = Description of Combined DNA/RNA Molecule: Synthetic oligonucleotide
  source 1..21: mol_type = other DNA
tctcaattgatctaaatgctt

SEQ ID NO: 115 - skipped

SEQ ID NO: 116 - DNA, 21 bp, synthetic construct
  misc_feature 1..21: note = Description of Artificial Sequence: Synthetic oligonucleotide
  misc_feature 1..21: note = Description of Combined DNA/RNA Molecule: Synthetic oligonucleotide
  source 1..21: mol_type = other DNA
ggttttaatggataaatcatt

SEQ ID NO: 117 - DNA, 21 bp, synthetic construct
  misc_feature 1..21: note = Description of Artificial Sequence: Synthetic oligonucleotide
  misc_feature 1..21: note = Description of Combined DNA/RNA Molecule: Synthetic oligonucleotide
  source 1..21: mol_type = other DNA
tgatttatccattaaaacctt

SEQ ID NO: 118 - skipped

SEQ ID NO: 119 - DNA, 21 bp, synthetic construct
  misc_feature 1..21: note = Description of Artificial Sequence: Synthetic oligonucleotide
  misc_feature 1..21: note = Description of Combined DNA/RNA Molecule: Synthetic oligonucleotide
  source 1..21: mol_type = other DNA
gactttgcagagcaatatttt

SEQ ID NO: 120 - DNA, 21 bp, synthetic construct
  misc_feature 1..21: note = Description of Artificial Sequence: Synthetic oligonucleotide
  misc_feature 1..21: note = Description of Combined DNA/RNA Molecule: Synthetic oligonucleotide
  source 1..21: mol_type = other DNA
aatattgctctgcaaagtctt

SEQ ID NO: 121 - skipped

SEQ ID NO: 122 - DNA, 21 bp, synthetic construct
  misc_feature 1..21: note = Description of Artificial Sequence: Synthetic oligonucleotide
  misc_feature 1..21: note = Description of Combined DNA/RNA Molecule: Synthetic oligonucleotide
  source 1..21: mol_type = other DNA
cttacgggtcatccaaaaatt

SEQ ID NO: 123 - DNA, 21 bp, synthetic construct
  misc_feature 1..21: note = Description of Artificial Sequence: Synthetic oligonucleotide
  misc_feature 1..21: note = Description of Combined DNA/RNA Molecule: Synthetic oligonucleotide
  source 1..21: mol_type = other DNA
tttttggatgacccgtaagtt

SEQ ID NO: 124 - skipped

SEQ ID NO: 125 - DNA, 21 bp, synthetic construct
  misc_feature 1..21: note = Description of Artificial Sequence: Synthetic oligonucleotide
  misc_feature 1..21: note = Description of Combined DNA/RNA Molecule: Synthetic oligonucleotide
  source 1..21: mol_type = other DNA
ggatcatctcaagtcttactt

SEQ ID NO: 126 - DNA, 21 bp, synthetic construct
  misc_feature 1..21: note = Description of Artificial Sequence: Synthetic oligonucleotide
  misc_feature 1..21: note = Description of Combined DNA/RNA Molecule: Synthetic oligonucleotide
  source 1..21: mol_type = other DNA
gtaagacttgagatgatcctt

SEQ ID NO: 127 - DNA, 20 bp, synthetic construct
  misc_feature 1..20: note = Description of Artificial Sequence: Synthetic oligonucleotide
  misc_feature 1..20: note = Description of Combined DNA/RNA Molecule: Synthetic oligonucleotide
  source 1..20: mol_type = other DNA
gcaaaggcgtgccaactcat

SEQ ID NO: 128 - RNA, 21 nt, synthetic construct
  modified_base 1: mod_base = OTHER; note = thymine
  modified_base 5..6: mod_base = OTHER; note = thymine
  modified_base 15..17: mod_base = OTHER; note = thymine
  modified_base 20..21: mod_base = OTHER; note = thymine
  misc_feature 1..21: note = Description of Artificial Sequence: Synthetic oligonucleotide
  source 1..21: mol_type = other RNA
tgagttggcacgcctttgctt

SEQ ID NO: 129 - DNA, 20 bp, synthetic construct
  misc_feature 1..20: note = Description of Artificial Sequence: Synthetic oligonucleotide
  misc_feature 1..20: note = Description of Combined DNA/RNA Molecule: Synthetic oligonucleotide
  source 1..20: mol_type = other DNA
ctatttggagagaaatcgat

SEQ ID NO: 130 - DNA, 21 bp, synthetic construct
  misc_feature 1..21: note = Description of Artificial Sequence: Synthetic oligonucleotide
  misc_feature 1..21: note = Description of Combined DNA/RNA Molecule: Synthetic oligonucleotide
  source 1..21: mol_type = other DNA
ggatcatctcaagtcttactt

SEQ ID NO: 131 - DNA, 21 bp, synthetic construct
  misc_feature 1..21: note = Description of Artificial Sequence: Synthetic oligonucleotide
  misc_feature 1..21: note = Description of Combined DNA/RNA Molecule: Synthetic oligonucleotide
  source 1..21: mol_type = other DNA
gtaagacttgagatgatcctt

SEQ ID NO: 132 - RNA, 21 nt, synthetic construct
  modified_base 1: mod_base = OTHER; note = thymine
  modified_base 5..7: mod_base = OTHER; note = thymine
  modified_base 9: mod_base = OTHER; note = thymine
  modified_base 11: mod_base = OTHER; note = thymine
  modified_base 17: mod_base = OTHER; note = thymine
  modified_base 20..21: mod_base = OTHER; note = thymine
  misc_feature 1..21: note = Description of Artificial Sequence: Synthetic oligonucleotide
  source 1..21: mol_type = other RNA
tcgatttctctccaaatagtt

SEQ ID NO: 133 - DNA, 20 bp, synthetic construct
  misc_feature 1..20: note = Description of Artificial Sequence: Synthetic oligonucleotide
  misc_feature 1..20: note = Description of Combined DNA/RNA Molecule: Synthetic oligonucleotide
  source 1..20: mol_type = other DNA
gcaaaggcgtgccaactcat

SEQ ID NO: 134 - DNA, 20 bp, synthetic construct
  misc_feature 1..20: note = Description of Artificial Sequence: Synthetic oligonucleotide
  misc_feature 1..20: note = Description of Combined DNA/RNA Molecule: Synthetic oligonucleotide
  source 1..20: mol_type = other DNA
ctatttggagagaaatcgat

SEQ ID NO: 135 - DNA, 22 bp, synthetic construct
  misc_feature 1..22: note = Description of Artificial Sequence: Synthetic oligonucleotide
  misc_feature 1..22: note = Description of Combined DNA/RNA Molecule: Synthetic oligonucleotide
  source 1..22: mol_type = other DNA
aacagtgttcttgctctataat

SEQ ID NO: 136 - RNA, 21 nt, synthetic construct
  modified_base 1: mod_base = OTHER; note = thymine
  modified_base 5..7: mod_base = OTHER; note = thymine
  modified_base 9: mod_base = OTHER; note = thymine
  modified_base 11: mod_base = OTHER; note = thymine
  modified_base 17: mod_base = OTHER; note = thymine
  modified_base 20..21: mod_base = OTHER; note = thymine
  misc_feature 1..21: note = Description of Artificial Sequence: Synthetic oligonucleotide
  source 1..21: mol_type = other RNA
tcgatttctctccaaatagtt

SEQ ID NO: 137 - DNA, 20 bp, synthetic construct
  misc_feature 1..20: note = Description of Artificial Sequence: Synthetic oligonucleotide
  misc_feature 1..20: note = Description of Combined DNA/RNA Molecule: Synthetic oligonucleotide
  source 1..20: mol_type = other DNA
gcaaaggcgtgccaactcat

SEQ ID NO: 138 - DNA, 20 bp, synthetic construct
  misc_feature 1..20: note = Description of Artificial Sequence: Synthetic oligonucleotide
  misc_feature 1..20: note = Description of Combined DNA/RNA Molecule: Synthetic oligonucleotide
  source 1..20: mol_type = other DNA
gcaaaggcgtgccaactcat

SEQ ID NO: 139 - RNA, 21 nt, synthetic construct
  modified_base 1: mod_base = OTHER; note = thymine
  modified_base 5..6: mod_base = OTHER; note = thymine
  modified_base 15..17: mod_base = OTHER; note = thymine
  modified_base 20..21: mod_base = OTHER; note = thymine
  misc_feature 1..21: note = Description of Artificial Sequence: Synthetic oligonucleotide
  source 1..21: mol_type = other RNA
tgagttggcacgcctttgctt

SEQ ID NO: 140 - DNA, 20 bp, synthetic construct
  misc_feature 1..20: note = Description of Artificial Sequence: Synthetic oligonucleotide
  misc_feature 1..20: note = Description of Combined DNA/RNA Molecule: Synthetic oligonucleotide
  source 1..20: mol_type = other DNA
ctatttggagagaaatcgat

SEQ ID NO: 141 - RNA, 21 nt, synthetic construct
  modified_base 1: mod_base = OTHER; note = thymine
  modified_base 5..7: mod_base = OTHER; note = thymine
  modified_base 9: mod_base = OTHER; note = thymine
  modified_base 11: mod_base = OTHER; note = thymine
  modified_base 17: mod_base = OTHER; note = thymine
  modified_base 20..21: mod_base = OTHER; note = thymine
  misc_feature 1..21: note = Description of Artificial Sequence: Synthetic oligonucleotide
  source 1..21: mol_type = other RNA
tcgatttctctccaaatagtt

SEQ ID NO: 142 - DNA, 22 bp, synthetic construct
  misc_feature 1..22: note = Description of Artificial Sequence: Synthetic oligonucleotide
  misc_feature 1..22: note = Description of Combined DNA/RNA Molecule: Synthetic oligonucleotide
  source 1..22: mol_type = other DNA
aacagtgttcttgctctataat

SEQ ID NO: 143 - RNA, 23 nt, synthetic construct
  modified_base 1..2: mod_base = OTHER; note = thymine
  modified_base 4: mod_base = OTHER; note = thymine
  modified_base 18: mod_base = OTHER; note = thymine
  modified_base 20..23: mod_base = OTHER; note = thymine
  misc_feature 1..23: note = Description of Artificial Sequence: Synthetic oligonucleotide
  source 1..23: mol_type = other RNA
ttatagagcaagaacactgtttt

SEQ ID NO: 144 - DNA, 20 bp, synthetic construct
  misc_feature 1..20: note = Description of Artificial Sequence: Synthetic oligonucleotide
  misc_feature 1..20: note = Description of Combined DNA/RNA Molecule: Synthetic oligonucleotide
  source 1..20: mol_type = other DNA
ctatttggagagaaatcgat

SEQ ID NO: 145 - DNA, 22 bp, synthetic construct
  misc_feature 1..22: note = Description of Artificial Sequence: Synthetic oligonucleotide
  misc_feature 1..22: note = Description of Combined DNA/RNA Molecule: Synthetic oligonucleotide
  source 1..22: mol_type = other DNA
aacagtgttcttgctctataat

SEQ ID NO: 146 - DNA, 21 bp, synthetic construct
  misc_feature 1..21: note = Description of Artificial Sequence: Synthetic oligonucleotide
  misc_feature 1..21: note = Description of Combined DNA/RNA Molecule: Synthetic oligonucleotide
  source 1..21: mol_type = other DNA
ggatcatctcaagtcttactt

SEQ ID NO: 147 - DNA, 21 bp, synthetic construct
  misc_feature 1..21: note = Description of Artificial Sequence: Synthetic oligonucleotide
  misc_feature 1..21: note = Description of Combined DNA/RNA Molecule: Synthetic oligonucleotide
  source 1..21: mol_type = other DNA
gtaagacttgagatgatcctt

SEQ ID NO: 148 - DNA, 21 bp, synthetic construct
  misc_feature 1..21: note = Description of Artificial Sequence: Synthetic oligonucleotide
  misc_feature 1..21: note = Description of Combined DNA/RNA Molecule: Synthetic oligonucleotide
  source 1..21: mol_type = other DNA
ggatcatctcaagtcttactt

SEQ ID NO: 149 - DNA, 21 bp, synthetic construct
  misc_feature 1..21: note = Description of Artificial Sequence: Synthetic oligonucleotide
  misc_feature 1..21: note = Description of Combined DNA/RNA Molecule: Synthetic oligonucleotide
  source 1..21: mol_type = other DNA
gtaagacttgagatgatcctt

SEQ ID NO: 150 - DNA, 21 bp, synthetic construct
  misc_feature 1..21: note = Description of Artificial Sequence: Synthetic oligonucleotide
  misc_feature 1..21: note = Description of Combined DNA/RNA Molecule: Synthetic oligonucleotide
  source 1..21: mol_type = other DNA
ggatcatctcaagtcttactt

SEQ ID NO: 151 - DNA, 21 bp, synthetic construct
  misc_feature 1..21: note = Description of Artificial Sequence: Synthetic oligonucleotide
  misc_feature 1..21: note = Description of Combined DNA/RNA Molecule: Synthetic oligonucleotide
  source 1..21: mol_type = other DNA
ggatcatctcaagtcttactt

SEQ ID NO: 152 - DNA, 21 bp, synthetic construct
  misc_feature 1..21: note = Description of Artificial Sequence: Synthetic oligonucleotide
  misc_feature 1..21: note = Description of Combined DNA/RNA Molecule: Synthetic oligonucleotide
  source 1..21: mol_type = other DNA
gtaagacttgagatgatcctt

SEQ ID NO: 153 - DNA, 21 bp, synthetic construct
  misc_feature 1..21: note = Description of Artificial Sequence: Synthetic oligonucleotide
  misc_feature 1..21: note = Description of Combined DNA/RNA Molecule: Synthetic oligonucleotide
  source 1..21: mol_type = other DNA
gtaagacttgagatgatcctt

SEQ ID NO: 154 - DNA, 21 bp, synthetic construct
  misc_feature 1..21: note = Description of Artificial Sequence: Synthetic oligonucleotide
  misc_feature 1..21: note = Description of Combined DNA/RNA Molecule: Synthetic oligonucleotide
  source 1..21: mol_type = other DNA
ggatcatctcaagtcttactt

SEQ ID NO: 155 - DNA, 21 bp, synthetic construct
  misc_feature 1..21: note = Description of Artificial Sequence: Synthetic oligonucleotide
  misc_feature 1..21: note = Description of Combined DNA/RNA Molecule: Synthetic oligonucleotide
  source 1..21: mol_type = other DNA
ggatcatctcaagtcttactt

SEQ ID NO: 156 - DNA, 21 bp, synthetic construct
  misc_feature 1..21: note = Description of Artificial Sequence: Synthetic oligonucleotide
  misc_feature 1..21: note = Description of Combined DNA/RNA Molecule: Synthetic oligonucleotide
  source 1..21: mol_type = other DNA
gtaagacttgagatgatcctt

SEQ ID NO: 157 - DNA, 21 bp, synthetic construct
  misc_feature 1..21: note = Description of Artificial Sequence: Synthetic oligonucleotide
  misc_feature 1..21: note = Description of Combined DNA/RNA Molecule: Synthetic oligonucleotide
  source 1..21: mol_type = other DNA
gtaagacttgagatgatcctt

SEQ ID NO: 158 - DNA, 21 bp, synthetic construct
  misc_feature 1..21: note = Description of Artificial Sequence: Synthetic oligonucleotide
  misc_feature 1..21: note = Description of Combined DNA/RNA Molecule: Synthetic oligonucleotide
  source 1..21: mol_type = other DNA
gtaagacttgagatgatcctt

SEQ ID NO: 159 - DNA, 21 bp, synthetic construct
  misc_feature 1..21: note = Description of Artificial Sequence: Synthetic oligonucleotide
  misc_feature 1..21: note = Description of Combined DNA/RNA Molecule: Synthetic oligonucleotide
  source 1..21: mol_type = other DNA
ggatcatctcaagtcttactt

SEQ ID NO: 160 - DNA, 21 bp, synthetic construct
  misc_feature 1..21: note = Description of Artificial Sequence: Synthetic oligonucleotide
  misc_feature 1..21: note = Description of Combined DNA/RNA Molecule: Synthetic oligonucleotide
  source 1..21: mol_type = other DNA
ggatcatctcaagtcttactt

SEQ ID NO: 161 - DNA, 21 bp, synthetic construct
  misc_feature 1..21: note = Description of Artificial Sequence: Synthetic oligonucleotide
  misc_feature 1..21: note = Description of Combined DNA/RNA Molecule: Synthetic oligonucleotide
  source 1..21: mol_type = other DNA
gtaagacttgagatgatcctt

SEQ ID NO: 162 - DNA, 21 bp, synthetic construct
  misc_feature 1..21: note = Description of Artificial Sequence: Synthetic oligonucleotide
  misc_feature 1..21: note = Description of Combined DNA/RNA Molecule: Synthetic oligonucleotide
  source 1..21: mol_type = other DNA
ggatcatctcaagtcttactt

SEQ ID NO: 163 - DNA, 21 bp, synthetic construct
  misc_feature 1..21: note = Description of Artificial Sequence: Synthetic oligonucleotide
  misc_feature 1..21: note = Description of Combined DNA/RNA Molecule: Synthetic oligonucleotide
  source 1..21: mol_type = other DNA
ggatcatctcaagtcttactt

SEQ ID NO: 164 - DNA, 21 bp, synthetic construct
  misc_feature 1..21: note = Description of Artificial Sequence: Synthetic oligonucleotide
  misc_feature 1..21: note = Description of Combined DNA/RNA Molecule: Synthetic oligonucleotide
  source 1..21: mol_type = other DNA
gtaagacttgagatgatcctt